European Patent Specification EP 3 822 363 B1, published September 6, 2023. Title: METHOD TO DETECT REPEAT SEQUENCE MOTIFS IN NUCLEIC ACID. Applicant: QUEST DIAGNOSTICS INVESTMENTS INCORPORATED. The sequence listing filed with the application follows.

SEQUENCE LISTING (113 sequences)

SEQ ID NO: 1 - DNA, 3240 bp, Homo sapiens
aatccatgtcccttaaagggcacagggtgtctccacagggccgcccaaaatctggtgagagagggcgtagacgcctcaccttctgcctctacgggtcacaaaagcctgggtcaccctggttgccactgttcctagttcaaagtcttcttctgtctaatccttcacccctattctcgccttccactccacctcccgctcagtcagactgcgctactttgaaccggaccaaaccaaaccaaaccaaaccaaaccaaaccagaccagacaccccctcccgcggaatcccagagaggccgaactgggataaccggatgcatttgatttcccacgccactgagtgcacctctgcagaaatgggcgttctggccctcgcgaggcagtgcgacctgtcaccgcccttcagccttcccgccctccaccaagcccgcgcacgcccggcccgcgcgtctgtctttcgacccggcaccccggccggttcccagcagcgcgcatgcgcgcgctcccaggccacttgaagagagagggcggggccgaggggctgagcccgcggggggagggaacagcgttgatcacgtgacgtggtttcagtgtttacacccgcagcgggccgggggttcggcctcagtcaggcgctcagctccgtttcggtttcacttccggtggagggccgcctctgagcgggcggcgggccgacggcgagcgcgggcggcggcggtgacggaggcgccgctgccagggggcgtgcggcagcgcggcggcggcggcggcggcggcggcggcggaggcggcggcggcggcggcggcggcggcggctgggcctcgagcgcccgcagcccacctctcgggggcgggctcccggcgctagcagggctgaagagaagatggaggagctggtggtggaagtgcggggctccaatggcgctttctacaaggtacttggctctagggcaggccccatcttcgcccttccttccctcccttttcttcttggtgtcggcgggaggcaggcccggggccctcttcccgagcaccgcgcctgggtgccagggcacgctcggcgggatgttgttgggagggaaggactggacttggggcctgttggaagcccctctccgactccgagaggccctagcgcctatcgaaatgagagaccagcgaggagagggttctctttcggcgccgagccccgccggggtgagctggggatgggcgagggccggcggcaggtactagagccgggcgggaagggccgaaatcggcgctaagtgacggcgatggcttattccccctttcctaaacatcatctcccagcgggatccgggcctgtcgtgtgggtagttgtggaggagcggggggcgcttcagccgggccgcctcctgcagcgccaagagggcttcaggtctcctttggcttctcttttccggtctagcattgggacttcggagagctccactgttctgggcgagggctgtgaagaaagagtagtaagaagcggtagtcggcaccaaatcacaatggcaactgatttttagtggcttctctttgtggatttcggaggagattttagatccaaaagtttcaggaagaccctaacatggcccagcagtgcattgaagaagttgatcatcgtgaatattcgcgtccccctttttgttaaacggggtaaattcaggaatgcacatgcttcagcgtctaaaaccattagcagcgctgctacttaaaaattgtgtgtgtgtgtttaagtttccaaagacctaaatatatgccatgaaacttcaggtaattaactgagagtatattattactagggcattttttttttaactgagcgaaaatatttttgtgcccctaagaacttgaccacatttcctttgaatttgtggtgttgcagtggactgaattgttgaggctttatataggcattcatgggtttactgtgctttttaaagttacaccattgcagatcaactaacacctttcagttttaaaaggaagatttacaaatttgatgtagcagtagtgcgtttgttggtatgtaggtgctgtataaattcatctataaattctcatttccttttgaatgtctataacctctttcaataatatcccaccttactacagtattttggcaatagaaggtgcgtgtggaaggaaggctggaaaatagctattagcagtgtccaacacaattcttaaatgtattgtagaatggcttgaatgtttcagacaggacacgtttggctataggaaaataaacaattgactttattctgtgtttaccaattttatgaagacatttggagatcagtatatttcataaatgagtaaagtatgtaaactgttccatactttgagcacaaagataaagccttttgctgtaaaaggaggcaaaaggtaaccccgcgtttatgttcttaacagtctcatgaatatgaaattgtttcagttgactctgcagtcaaaattttaatttcattgattttattgatccataatttcttctggtgagtttgcgtagaatcgttcacggtcctagattagtggttttggtcactagatttctggcactaataactataatacatatacatatatatgtgtgagtaacggctaatggttaggcaagattttgattgacctgtgatataaacttagattggatgccactaaagtttgcttatcacagagggcaagtagcacattatggccttgaagtacttattgttctcttccagcaacttatgatttgctccagtgattttgcttgcacactgactggaatataagaaatgccttctatttttgctattaattccctccttttttgttttgttttgtaacgaagttgtttaacttgaaggtgaatgaagaataggttggttgccccttagttccctgaggagaaatgttaatacttgaacaagtgtgtgtcagacaaattgctgttatgtttatttaattaagtttgatttctaagaaaatctcaaatggtctgcactgatggaagaacagtttctgtaacaaaaaagcttgaaatttttatatgacttataatactgctgtgagttttaaaagtaaagcaaaagtaaactgagttgcttgtccagtgggatggacaggaaagatgtgaaataaaaaccaatgaaaaatgaactgctgtggagaagtgttacatttatggaaaaagaaataggaaccttgttcatcaaattgatagaaaagcttttaaaactaaacaaa

SEQ ID NO: 2 - DNA, 48 bp, Artificial Sequence
  Description of Artificial Sequence: Synthetic primer
tgtaaaacgacggccagtgctcagctccgtttcggtttcacttccggt

SEQ ID NO: 3 - DNA, 41 bp, Artificial Sequence
  Description of Artificial Sequence: Synthetic primer
caggaaacagctatgaccctcgaggcccagccgccgccgcc

SEQ ID NO: 4 - DNA, 29 bp, Artificial Sequence
  Description of Artificial Sequence: Synthetic primer
caggaaacagctatgaccccgccgccgcc

SEQ ID NO: 5 - DNA, 28 bp, Artificial Sequence
  Description of Artificial Sequence: Synthetic primer
caggaaacagctatgacccgccgccgcc

SEQ ID NO: 6 - DNA, 35 bp, Artificial Sequence
  Description of Artificial Sequence: Synthetic primer
caggaaacagctatgaccccgccgdcgccgccgcc

SEQ ID NO: 7 - DNA, 48 bp, Artificial Sequence
  Description of Artificial Sequence: Synthetic primer
caggaaacagctatgaccccgccgccgccgccgccgccgccgccgccg

SEQ ID NO: 8 - DNA, 39 bp, Artificial Sequence
  Description of Artificial Sequence: Synthetic primer
caggaaacagctatgaccccgccgccgccgccgccgccg

SEQ ID NO: 9 - DNA, 47 bp, Artificial Sequence
  Description of Artificial Sequence: Synthetic primer
caggaaacagctatgaccccgccgccgccgccgccgccgccgccgcc

SEQ ID NO: 10 - DNA, 38 bp, Artificial Sequence
  Description of Artificial Sequence: Synthetic primer
caggaaacagctatgaccccgccgccgccgccgccgcc

SEQ ID NO: 11 - DNA, 18 bp, Artificial Sequence
  Description of Artificial Sequence: Synthetic primer
caggaaacagctatgacc

SEQ ID NO: 12 - DNA, 30 bp, Artificial Sequence
  Description of Artificial Sequence: Synthetic primer
gctcagctccgtttcggtttcacttccggt

SEQ ID NO: 13 - DNA, 35 bp, Artificial Sequence
  Description of Artificial Sequence: Synthetic primer
agccccgcacttccactttcggtttcacttccggt

SEQ ID NO: 14 - DNA, 10 bp, Artificial Sequence
  Description of Artificial Sequence: Synthetic primer
cgccgccgcc

SEQ ID NO: 15 - DNA, 13 bp, Artificial Sequence
  Description of Artificial Sequence: Synthetic primer
ccgccgaccgccg

SEQ ID NO: 16 - DNA, 13 bp, Artificial Sequence
  Description of Artificial Sequence: Synthetic primer
ccgccgtccgccg

SEQ ID NO: 17 - DNA, 13 bp, Artificial Sequence
  Description of Artificial Sequence: Synthetic primer
ccgccggccgccg

SEQ ID NO: 18 - DNA, 13 bp, Artificial Sequence
  Description of Artificial Sequence: Synthetic primer
ccgccgcccgccg

SEQ ID NO: 19 - DNA, 19 bp, Artificial Sequence
  Description of Artificial Sequence: Synthetic primer
cgccgccgacgccgccgcc

SEQ ID NO: 20 - DNA, 19 bp, Artificial Sequence
  Description of Artificial Sequence: Synthetic primer
cgccgccgtcgccgccgcc

SEQ ID NO: 21 - DNA, 19 bp, Artificial Sequence
  Description of Artificial Sequence: Synthetic primer
cgccgccggcgccgccgcc

SEQ ID NO: 22 - DNA, 17 bp, Artificial Sequence
  Description of Artificial Sequence: Synthetic primer
cgccgccgcccgccgcc

SEQ ID NO: 23 - DNA, 18 bp, Artificial Sequence
  Description of Artificial Sequence: Synthetic primer
ctcgaggcccagccgccg

SEQ ID NO: 24 - DNA, 21 bp, Artificial Sequence
  Description of Artificial Sequence: Synthetic primer
ctcgaggcccagccgtcgccg

SEQ ID NO: 25 - DNA, 21 bp, Artificial Sequence
  Description of Artificial Sequence: Synthetic primer
ctcgaggcccagccgacgccg

SEQ ID NO: 26 - DNA, 21 bp, Artificial Sequence
  Description of Artificial Sequence: Synthetic primer
ctcgaggcccagccggcgccg

SEQ ID NO: 27 - DNA, 23 bp, Artificial Sequence
  Description of Artificial Sequence: Synthetic primer
caggaaacagctatgacccgccg

SEQ ID NO: 28 - DNA, 26 bp, Artificial Sequence
  Description of Artificial Sequence: Synthetic primer
caggaaacagctatgacgccgccgcc

SEQ ID NO: 29 - DNA, 30 bp, Artificial Sequence
  Description of Artificial Sequence: Synthetic primer
caggaaacagctatgacccgccgaccgccg

SEQ ID NO: 30 - DNA, 30 bp, Artificial Sequence
  Description of Artificial Sequence: Synthetic primer
caggaaacagctatgacccgccgtccgccg

SEQ ID NO: 31 - DNA, 30 bp, Artificial Sequence
  Description of Artificial Sequence: Synthetic primer
caggaaacagctatgacccgccggccgccg

SEQ ID NO: 32 - DNA, 30 bp, Artificial Sequence
  Description of Artificial Sequence: Synthetic primer
caggaaacagctatgacccgccgcccgccg

SEQ ID NO: 33 - DNA, 35 bp, Artificial Sequence
  Description of Artificial Sequence: Synthetic primer
caggaaacagctatgacgccgccgacgccgccgcc

SEQ ID NO: 34 - DNA, 35 bp, Artificial Sequence
  Description of Artificial Sequence: Synthetic primer
caggaaacagctatgacgccgccgtcgccgccgcc

SEQ ID NO: 35 - DNA, 35 bp, Artificial Sequence
  Description of Artificial Sequence: Synthetic primer
caggaaacagctatgacgccgccggcgccgccgcc

SEQ ID NO: 36 - DNA, 33 bp, Artificial Sequence
  Description of Artificial Sequence: Synthetic primer
caggaaacagctatgacgccgccgcccgccgcc

SEQ ID NO: 37 - DNA, 34 bp, Artificial Sequence
  Description of Artificial Sequence: Synthetic primer
caggaaacagctatgacctcgaggcccaccgccg

SEQ ID NO: 38 - DNA, 41 bp, Artificial Sequence
  Description of Artificial Sequence: Synthetic primer
caggaaacagctatgacctcgaggcccagccgtcgccgccg

SEQ ID NO: 39 - DNA, 41 bp, Artificial Sequence
  Description of Artificial Sequence: Synthetic primer
caggaaacagctatgacctcgaggcccagccgacgccgccg

SEQ ID NO: 40 - DNA, 41 bp, Artificial Sequence
  Description of Artificial Sequence: Synthetic primer
caggaaacagctatgacctcgaggcccagccggcgccgccg

SEQ ID NO: 41 - DNA, 10 bp, Artificial Sequence
  Description of Artificial Sequence: Synthetic primer
cgcggcggcg

SEQ ID NO: 42 - DNA, 13 bp, Artificial Sequence
  Description of Artificial Sequence: Synthetic primer
cggcggacggcgg

SEQ ID NO: 43 - DNA, 13 bp, Artificial Sequence
  Description of Artificial Sequence: Synthetic primer
cggcggtcggcgg

SEQ ID NO: 44 - DNA, 13 bp, Artificial Sequence
  Description of Artificial Sequence: Synthetic primer
cggcgggcggcgg

SEQ ID NO: 45 - DNA, 13 bp, Artificial Sequence
  Description of Artificial Sequence: Synthetic primer
cggcggccggcgg

SEQ ID NO: 46 - DNA, 19 bp, Artificial Sequence
  Description of Artificial Sequence: Synthetic primer
ggcggcggaggcggcggcg

SEQ ID NO: 47 - DNA, 19 bp, Artificial Sequence
  Description of Artificial Sequence: Synthetic primer
ggcggcggtggcggcggcg

SEQ ID NO: 48 - DNA, 19 bp, Artificial Sequence
  Description of Artificial Sequence: Synthetic primer
ggcggcgggggcggcggcg

SEQ ID NO: 49 - DNA, 17 bp, Artificial Sequence
  Description of Artificial Sequence: Synthetic primer
ggcggcggccggcggcg

SEQ ID NO: 50 - DNA, 18 bp, Artificial Sequence
  Description of Artificial Sequence: Synthetic primer
  modified_base (6)..(6): Inosine
cgtgcngcagcgcggcgg

SEQ ID NO: 51 - DNA, 21 bp, Artificial Sequence
  Description of Artificial Sequence: Synthetic primer
  modified_base (6)..(6): Inosine
cgtgcngcagcgcggtggcgg

SEQ ID NO: 52 - DNA, 21 bp, Artificial Sequence
  Description of Artificial Sequence: Synthetic primer
  modified_base (6)..(6): Inosine
cgtgcngcagcgcggaggcgg

SEQ ID NO: 53 - DNA, 21 bp, Artificial Sequence
  Description of Artificial Sequence: Synthetic primer
  modified_base (6)..(6): Inosine
cgtgcngcagcgcgggggcgg

SEQ ID NO: 54 - DNA, 23 bp, Artificial Sequence
  Description of Artificial Sequence: Synthetic primer
caggaaacagctatgaccggcgg

SEQ ID NO: 55 - DNA, 25 bp, Artificial Sequence
  Description of Artificial Sequence: Synthetic primer
caggaaacagctatgaccggcggcg

SEQ ID NO: 56 - DNA, 30 bp, Artificial Sequence
  Description of Artificial Sequence: Synthetic primer
caggaaacagctatgaccggcggacggcgg

SEQ ID NO: 57 - DNA, 30 bp, Artificial Sequence
  Description of Artificial Sequence: Synthetic primer
caggaaacagctatgaccggcggtcggcgg

SEQ ID NO: 58 - DNA, 30 bp, Artificial Sequence
  Description of Artificial Sequence: Synthetic primer
caggaaacagctatgaccggcggccggcgg

SEQ ID NO: 59 - DNA, 30 bp, Artificial Sequence
  Description of Artificial Sequence: Synthetic primer
caggaaacagctatgaccggcgggcggcgg

SEQ ID NO: 60 - DNA, 35 bp, Artificial Sequence
  Description of Artificial Sequence: Synthetic primer
caggaaacagctatgacccggcggaggcggcggcg

SEQ ID NO: 61 - DNA, 35 bp, Artificial Sequence
  Description of Artificial Sequence: Synthetic primer
caggaaacagctatgacccggcggtggcggcggcg

SEQ ID NO: 62 - DNA, 35 bp, Artificial Sequence
  Description of Artificial Sequence: Synthetic primer
caggaaacagctatgacccggcgggggcggcggcg

SEQ ID NO: 63 - DNA, 33 bp, Artificial Sequence
  Description of Artificial Sequence: Synthetic primer
caggaaacagctatgacccggcggccggcggcg

SEQ ID NO: 64 - DNA, 33 bp, Artificial Sequence
  Description of Artificial Sequence: Synthetic primer
caggaaacagctatgacccggcggtcggcggcg

SEQ ID NO: 65 - DNA, 33 bp, Artificial Sequence
  Description of Artificial Sequence: Synthetic primer
caggaaacagctatgacccggcgggcggcggcg

SEQ ID NO: 66 - DNA, 33 bp, Artificial Sequence
  Description of Artificial Sequence: Synthetic primer
caggaaacagctatgacccggcggacggcggcg

SEQ ID NO: 67 - DNA, 42 bp, Artificial Sequence
  Description of Artificial Sequence: Synthetic primer
  modified_base (24)..(24): Inosine
caggaaacagctatgacccgtgcngcagcgcggtggcggcgg

SEQ ID NO: 68 - DNA, 42 bp, Artificial Sequence
  Description of Artificial Sequence: Synthetic primer
  modified_base (24)..(24): Inosine
caggaaacagctatgacccgtgcngcagcgcggaggcggcgg

SEQ ID NO: 69 - DNA, 42 bp, Artificial Sequence
  Description of Artificial Sequence: Synthetic primer
  modified_base (24)..(24): Inosine
caggaaacagctatgacccgtgcngcagcgcgggggcggcgg

SEQ ID NO: 70 - DNA, 20 bp, Artificial Sequence
  Description of Artificial Sequence: Synthetic oligonucleotide
taatacgactcactataggg

SEQ ID NO: 71 - DNA, 44 bp, Artificial Sequence
  Description of Artificial Sequence: Synthetic primer
caggaaacagctatgaccctcgaggcccagccgccgccgccgcc

SEQ ID NO: 72 - DNA, 47 bp, Artificial Sequence
  Description of Artificial Sequence: Synthetic primer
caggaaacagctatgaccctcgaggcccagccgccgccgccgccgcc

SEQ ID NO: 73 - DNA, 38 bp, Artificial Sequence
  Description of Artificial Sequence: Synthetic primer
caggaaacagctatgaccctcgaggcccagccgccgcc

SEQ ID NO: 74 - DNA, 36 bp, Artificial Sequence
  Description of Artificial Sequence: Synthetic primer
caggaaacagctatgaccctcgaggcccagccgccg

SEQ ID NO: 75 - DNA, 479 bp, Homo sapiens
cgccgcctgtgcagccgctgccgccgccgccgccgccgccgccgccgccgccgccgccgccgccgctgccgccccggctgccgcgccgcgccgctgcctctgccccggccgcccccgccgccgctgccgccgccggcccgcagccagccaggcgggcggcccagcccgcctgagcccgcagcggctgccgccgcagcgtcgggtcgctgggtgcgcgggctaccgcggaccgagcggacccgagtgggcgaccaggcgcttgcccgcccagtgccactgccgccgcttcctcgccggagcacaggaccagacacctccagcgcccgctgctgctgccgatgcggcccggacacttttagctgggcgggagggctggagagccgggggccgccgagaaccgccagcgagctgtgccgagagccgcgccgacccgctgcgatcagggacaggcgcccgcccgccgccgccgcctggccgct

SEQ ID NO: 76 - DNA, 20 bp, Artificial Sequence
  Description of Artificial Sequence: Synthetic primer
cgccgcctgtgcagccgctg

SEQ ID NO: 77 - DNA, 20 bp, Artificial Sequence
  Description of Artificial Sequence: Synthetic primer
gccccggctgccgcgccgcg

SEQ ID NO: 78 - DNA, 45 bp, Artificial Sequence
  Description of Artificial Sequence: Synthetic primer
  misc_feature (1)..(45): This region may encompass 1 to 15 "ccg" repeating units
ccgccgccgccgccgccgccgccgccgccgccgccgccgccgccg

SEQ ID NO: 79 - DNA, 17 bp, Artificial Sequence
  Description of Artificial Sequence: Synthetic primer
ccgccgdcgccgccgcc

SEQ ID NO: 80 - DNA, 19 bp, Artificial Sequence
  Description of Artificial Sequence: Synthetic primer
cgccgccgdcgccgccgcc

SEQ ID NO: 81 - DNA, 15 bp, Artificial Sequence
  Description of Artificial Sequence: Synthetic primer
ccgccgdcgccgccg

SEQ ID NO: 82 - DNA, 18 bp, Artificial Sequence
  Description of Artificial Sequence: Synthetic primer
cgccgccgdcgccgccgc

SEQ ID NO: 83 - DNA, 17 bp, Artificial Sequence
  Description of Artificial Sequence: Synthetic primer
gcggcggdggcggcggc

SEQ ID NO: 84 - DNA, 13 bp, Artificial Sequence
  Description of Artificial Sequence: Synthetic primer
  modified_base (7)..(7): a, c, t or g
ccgccgnccgccg

SEQ ID NO: 85 - DNA, 17 bp, Artificial Sequence
  Description of Artificial Sequence: Synthetic primer
  modified_base (9)..(9): a, c, t or g
cgccgccgnccgccgcc

SEQ ID NO: 86 - DNA, 16 bp, Artificial Sequence
  Description of Artificial Sequence: Synthetic primer
  modified_base (8)..(8): a, c, t or g
gccgccgnccgccgcc

SEQ ID NO: 87 - DNA, 16 bp, Artificial Sequence
  Description of Artificial Sequence: Synthetic primer
  modified_base (9)..(9): a, c, t or g
cgccgccgnccgccgc

SEQ ID NO: 88 - DNA, 26 bp, Artificial Sequence
  Description of Artificial Sequence: Synthetic primer
ccgccgdcgccgccgdcgccgccgcc

SEQ ID NO: 89 - DNA, 28 bp, Artificial Sequence
  Description of Artificial Sequence: Synthetic primer
cgccgccgdcgccgccgdcgccgccgcc

SEQ ID NO: 90 - DNA, 20 bp, Artificial Sequence
  Description of Artificial Sequence: Synthetic primer
  modified_base (7)..(7): a, c, t or g
  modified_base (14)..(14): a, c, t or g
ccgccgnccgccgnccgccg

SEQ ID NO: 91 - DNA, 22 bp, Artificial Sequence
  Description of Artificial Sequence: Synthetic primer
  modified_base (7)..(7): a, c, t or g
  modified_base (14)..(14): a, c, t or g
ccgccgnccgccgnccgccgcc

SEQ ID NO: 92 - DNA, 24 bp, Artificial Sequence
  Description of Artificial Sequence: Synthetic primer
  modified_base (9)..(9): a, c, t or g
  modified_base (16)..(16): a, c, t or g
cgccgccgnccgccgnccgccgcc

SEQ ID NO: 93 - DNA, 11 bp, Artificial Sequence
  Description of Artificial Sequence: Synthetic primer
  modified_base (6)..(6): a, c, t or g
cgccgnccgcc

SEQ ID NO: 94 - DNA, 10 bp, Artificial Sequence
  Description of Artificial Sequence: Synthetic primer
  modified_base (5)..(5): a, c, t or g
gccgnccgcc

SEQ ID NO: 95 - DNA, 10 bp, Artificial Sequence
  Description of Artificial Sequence: Synthetic primer
cgccgccgcc

SEQ ID NO: 96 - DNA, 45 bp, Artificial Sequence
  Description of Artificial Sequence: Synthetic primer
  misc_feature (1)..(45): This region may encompass 1 to 15 "cgg" repeating units
cggcggcggcggcggcggcggcggcggcggcggcggcggcggcgg

SEQ ID NO: 97 - DNA, 17 bp, Artificial Sequence
  Description of Artificial Sequence: Synthetic primer
cggcggdggcggcggcg

SEQ ID NO: 98 - DNA, 19 bp, Artificial Sequence
  Description of Artificial Sequence: Synthetic primer
ggcggcggdggcggcggcg

SEQ ID NO: 99 - DNA, 15 bp, Artificial Sequence
  Description of Artificial Sequence: Synthetic primer
cggcggdggcggcgg

SEQ ID NO: 100 - DNA, 18 bp, Artificial Sequence
  Description of Artificial Sequence: Synthetic primer
ggcggcggdggcggcggc

SEQ ID NO: 101 - DNA, 17 bp, Artificial Sequence
  Description of Artificial Sequence: Synthetic primer
gcggcggdggcggcggc

SEQ ID NO: 102 - DNA, 13 bp, Artificial Sequence
  Description of Artificial Sequence: Synthetic primer
  modified_base (7)..(7): a, c, t or g
cggcggncggcgg

SEQ ID NO: 103 - DNA, 17 bp, Artificial Sequence
  Description of Artificial Sequence: Synthetic primer
  modified_base (9)..(9): a, c, t or g
ggcggcggncggcggcg

SEQ ID NO: 104 - DNA, 16 bp, Artificial Sequence
  Description of Artificial Sequence: Synthetic primer
  modified_base (8)..(8): a, c, t or g
gcggcggncggcggcg

SEQ ID NO: 105 - DNA, 15 bp, Artificial Sequence
  Description of Artificial Sequence: Synthetic primer
  modified_base (8)..(8): a, c, t or g
gcggcggncggcggc

SEQ ID NO: 106 - DNA, 26 bp, Artificial Sequence
  Description of Artificial Sequence: Synthetic primer
cggcggdggcggcggdggcggcggcg

SEQ ID NO: 107 - DNA, 28 bp, Artificial Sequence
  Description of Artificial Sequence: Synthetic primer
ggcggcggdggcggcggdggcggcggcg

SEQ ID NO: 108 - DNA, 20 bp, Artificial Sequence
  Description of Artificial Sequence: Synthetic primer
  modified_base (7)..(7): a, c, t or g
  modified_base (14)..(14): a, c, t or g
cggcggncggcggncggcgg

SEQ ID NO: 109 - DNA, 22 bp, Artificial Sequence
  Description of Artificial Sequence: Synthetic primer
  modified_base (7)..(7): a, c, t or g
  modified_base (14)..(14): a, c, t or g
cggcggncggcggncggcggcg

SEQ ID NO: 110 - DNA, 24 bp, Artificial Sequence
  Description of Artificial Sequence: Synthetic primer
  modified_base (9)..(9): a, c, t or g
  modified_base (16)..(16): a, c, t or g
ggcggcggncggcggncggcggcg

SEQ ID NO: 111 - DNA, 11 bp, Artificial Sequence
  Description of Artificial Sequence: Synthetic primer
  modified_base (6)..(6): a, c, t or g
ggcggncggcg

SEQ ID NO: 112 - DNA, 10 bp, Artificial Sequence
  Description of Artificial Sequence: Synthetic primer
  modified_base (5)..(5): a, c, t or g
gcggncggcg

SEQ ID NO: 113 - DNA, 10 bp, Artificial Sequence
  Description of Artificial Sequence: Synthetic primer
ggcggcggcg